European Patent Specification EP 3 978 601 B1, published February 26, 2025. Title: Recombinant Oncolytic Virus, Preparation Method Therefor, Use Thereof and Medicine Thereof. Applicant: ZETANG WU. The sequence listing filed with the application follows.

SEQUENCE LISTING (8 sequences)

SEQ ID NO: 1 - DNA, 22 bp, Artificial sequence
  The base sequence of the target sequence
caagctgaccctgaagttcata

SEQ ID NO: 2 - RNA, 21 nt, Artificial sequence
  The base sequence of the first interfering RNA
augaacuucagggucagcuug

SEQ ID NO: 3 - RNA, 22 nt, Artificial sequence
  The sequence of the second interfering RNA
cuugccugucuaacucgcuagu

SEQ ID NO: 4 - RNA, 25 nt, Artificial sequence
  The base sequence of the third interfering RNA
cuugcugaauacuugguccuuggug

SEQ ID NO: 5 - DNA, 2679 bp, Artificial sequence
  The base sequence of the DNA fragment A
aaataactcgagctgcgggcgctgttgttccatcatcctgtcgggcatcgcaatgcgattgtgttatatcgccgtggtggccggggtggtgctcgtggcgcttcactacgagcaggagatccagaggcgcctgtttgatgtatgacgtcacatccaggccggcggaaaccggaacggcatatgcaaactggaaactgtcctgtcttggggcccacccacccgacgcgtcatatgtaaatgaaaatcgttcccccgaggccatgtgtagcctggatcccaacgaccccgcccatgggtcccaattggccgtcccgttaccaagaccaacccagccagcgtatccacccccgcccgggtccccgcggaagcggaacggtgtatgtgatatgctaattaaatacatgccacgtacttatggtgtctgattggtccttgtctgtgccggaggtggggcgggggccccgcccggggggcggaactaggaggggtttgggagagccggccccggcaccacgggtataaggacatccaccacccggccggtggtggtgtgcagccgtgttccaaccacggtcgttgacattgattattgactagttattaatagtaatcaattacggggtcattagttcatagcccatatatggagttccgcgttacataacttacggtaaatggcccgcctggctgaccgcccaacgacccccgcccattgacgtcaataatgacgtatgttcccatagtaacgccaatagggactttccattgacgtcaatgggtggactatttacggtaaactgcccacttggcagtacatcaagtgtatcatatgccaagtacgccccctattgacgtcaatgacggtaaatggcccgcctggcattatgcccagtacatgaccttatgggactttcctacttggcagtacatctacgtattagtcatcgctattaccatggtgatgcggttttggcagtacatcaatgggcgtggatagcggtttgactcacggggatttccaagtctccaccccattgacgtcaatgggagtttgttttggcaccaaaatcaacgggactttccaaaatgtcgtaacaactccgccccattgacgcaaatgggcggtaggcgtgtacggtgggaggtctatataagcagagctctctggctaactgccaccatggtgagcaagggcgaggagctgttcaccggggtggtgcccatcctggtcgagctggacggcgacgtaaacggccacaagttcagcgtgtccggcgagggcgagggcgatgccacctacggcaagctgaccctgaagttcatctgcaccaccggcaagctgcccgtgccctggcccaccctcgtgaccaccctgacctacggcgtgcagtgcttcagccgctaccccgaccacatgaagcagcacgacttcttcaagtccgccatgcccgaaggctacgtccaggagcgcaccatcttcttcaaggacgacggcaactacaagacccgcgccgaggtgaagttcgagggcgacaccctggtgaaccgcatcgagctgaagggcatcgacttcaaggaggacggcaacatcctggggcacaagctggagtacaactacaacagccacaacgtctatatcatggccgacaagcagaagaacggcatcaaggtgaacttcaagatccgccacaacatcgaggacggcagcgtgcagctcgccgaccactaccagcagaacacccccatcggcgacggccccgtgctgctgcccgacaaccactacctgagcacccagtccgccctgagcaaagaccccaacgagaagcgcgatcacatggtcctgctggagttcgtgaccgccgccgggatcactctcggcatggacgagctgtacaagtaacgggcctcgactgtgccttctagttgccagccatctgttgtttgcccctcccccgtgccttccttgaccctggaaggtgccactcccactgtcctttcctaataaaatgaggaaattgcatcgcattgtctgagtaggtgtcattctattctggggggtggggtggggcaggacagcaagggggaggattgggaagacaatagcaggcatgctggggatgcggtgggctctatggcttctgaggtacaataaaaacaaaacatttcaaacaaatcgccccacgtgttgtccttctttgctcatggccggcggggcgtgggtcacggcagatggcgggggtgggcccggcgtacggcctgggtgggcggagggaactaacccaacgtataaatccgtccccgctccaaggccggtgtcatagtgcccttaggagcttcccgcccgggcgcatccccccttttgcactatgacagcgacccccctcaccaacctgttcttacgggccccggacataacccacgtggcccccccttactgcctcaacgccacctggcaggccgaaacggccatgcacaccagcaaaacggactccgcttgcgtggccgtgcggagttacctggtccgcgcctcctgtgagaccagcggcacaatccactgctttttctttgcggtatacaaggacacccaccatacccctccgctgattaccgagctccgcaactttgcggacctggttaaccacccgccggtcctacgcgaactggtcgaagctttttata

SEQ ID NO: 6 - DNA, 3338 bp, Artificial sequence
  The base sequence of the DNA fragment B
cccaaactcgagctgcgggcgctgttgttccatcatcctgtcgggcatcgcaatgcgattgtgttatatcgccgtggtggccggggtggtgctcgtggcgcttcactacgagcaggagatccagaggcgcctgtttgatgtatgacgtcacatccaggccggcggaaaccggaacggcatatgcaaactggaaactgtcctgtcttggggcccacccacccgacgcgtcatatgtaaatgaaaatcgttcccccgaggccatgtgtagcctggatcccaacgaccccgcccatgggtcccaattggccgtcccgttaccaagaccaacccagccagcgtatccacccccgcccgggtccccgcggaagcggaacggtgtatgtgatatgctaattaaatacatgccacgtacttatggtgtctgattggtccttgtctgtgccggaggtggggcgggggccccgcccggggggcggaactaggaggggtttgggagagccggccccggcaccacgggtataaggacatccaccacccggccggtggtggtgtgcagccgtgttccaaccacggtcacgcttcggtgcctctccccgattcgggcccggtcgcttgctaccggtgcgccaccaccagaggccatatccgacaccccagccccgacggcagccgacagcccggtcatggcgactgacattgatatgctaattgacctcggcctggacctctccgacagcgatctggacgaggacccccccgagccggcggagagccgccgcgacgacctggaatcggacagcaacggggagtgttcctcgtcggacgaggacatggaagacccccacggagaggacggaccggagccgatactcgacgccgctcgcccggcggtccgcccgtctcgtccagaagaccccggcgtacccagcacccagacgcctcgtccgacggagcggcagggccccaacgatcctcaaccagcgccccacagtgtgtggtcgcgcctcggggcccggcgaccgtcttgctcccccgagcggcacgggggcaaggtggcccgcctccaacccccaccgaccaaagcccagcctgcccgcggcggacgccgtgggcgtcgcaggggtcggggtcgcggtggtcccggggccgccgatggtttgtcggacccccgccggcgtgcccccagaaccaatcgcaacccggggggaccccgccccggggcggggtggacggacggccccggcgccccccatggcgaggcgtggcgcggaagtgagcagcccgacccacccggaggcccgcggacacggagcgtgcgccaagcaccccccccgctaatgacgctggcgattgcccccccgcccgcggacccccgcgccccggccccggagcgaaaggcgcccgccgccgacaccatcgacgccaccacgcggttggtcctgcgctccatctccgagcgcgcggcggtcgaccgcatcagcgagagcttcggccgcagcgcacaggtcatgcacgacccctttggggggcagccgtttcccgccgcgaatagcccctgggccccggtgctggcgggccaaggagggccctttgacgccgagaccagacgggtctcctgggaaaccttggtcgcccacggcccgagcctctatcgcacttttgccggcaatcctcgggccgcatcgaccgccaaggccatgcgcgactgcgtgctgcgccaagaaaatttcatcgaggcgctggcctccgccgacgagacgctggcgtggtgcaagatgtgcatccaccacaacctgccgctgcgcccccaggaccccattatcgggacggccgcggcggtgctggataacctcgccacgcgcctgcggccctttctccagtgctacctgaaggcgcgaggcctgtgcggcctggacgaactgtgttcgcggcggcgtctggcggacattaaggacattgcatccttcgtgtttgtcattctggccaggctcgccaaccgcgtcgagcgtggcgtcgcggagatcgactacgcgacccttggtgtcggggtcggagagaagatgcatttctacctccccggggcctgcatggcgggcctgatcgaaatcctagacacgcaccgccaggagtgttcgagtcgtgtctgcgagttgacggccagtcacatcgtcgcccccccgtacgtgcacggcaaatatttttattgcaactccctgttttaggatcgcaagctgaccctgaagttcatagtccaagctgaccctgaagttcatacgtccacatgaagcagcacgacttctgaccacatgaagcagcacgacttgatccagacatgataagatacattgatgagtttggacaaaccacaactagaatgcagtgaaaaaaatgctttatttgtgaaatttgtgatgctattgctttatttgtaaccattataagctgcaataaacaagttaacaacaacaattgcattcattttatgtttcaggttcagggggaggtgtgggaggttttttaaagcaagtaaaacctctacaaatgtggtatggctgattatgatcctgcaagcctcgtcgtcctggccggaccacgctatctgtgcaaggtccccggccccggacgcgcgctccatgagcagagcgcccgccgccgaggcgaagactcgggcggcgccctgcccgtcccaccaggtcaacaggcggtaaccggcctcttcatcgggaatgcgcgcgaccttcagcatcgccggcatgtccccctggcggacgggaagtatccagctcgaccaagctgttttaagcttgtacaataaaaacaaaacatttcaaacaaatcgccccacgtgttgtccttctttgctcatggccggcggggcgtgggtcacggcagatggcgggggtgggcccggcgtacggcctgggtgggcggagggaactaacccaacgtataaatccgtccccgctccaaggccggtgtcatagtgcccttaggagcttcccgcccgggcgcatccccccttttgcactatgacagcgacccccctcaccaacctgttcttacgggccccggacataacccacgtggcccccccttactgcctcaacgccacctggcaggccgaaacggccatgcacaccagcaaaacggactccgcttgcgtggccgtgcggagttacctggtccgcgcctcctgtgagaccagcggcacaatccactgctttttctttgcggtatacaaggacacccaccatacccctccgctgattaccgagctccgcaactttgcggacctggttaaccacccgccggtcctacgcgaactgctcgaggggaaa

SEQ ID NO: 7 - DNA, 2622 bp, Artificial sequence
  The base sequence of the DNA fragment C
aataatataagcttgttgacattgattattgactagttattaatagtaatcaattacggggtcattagttcatagcccatatatggagttccgcgttacataacttacggtaaatggcccgcctggctgaccgcccaacgacccccgcccattgacgtcaataatgacgtatgttcccatagtaacgccaatagggactttccattgacgtcaatgggtggagtatttacggtaaactgcccacttggcagtacatcaagtgtatcatatgccaagtacgccccctattgacgtcaatgacggtaaatggcccgcctggcattatgcccagtacatgaccttatgggactttcctacttggcagtacatctacgtattagtcatcgctattaccatggtgatgcggttttggcagtacatcaatgggcgtggatagcggtttgactcacggggatttccaagtctccaccccattgacgtcaatgggagtttgttttggcaccaaaatcaacgggactttccaaaatgtcgtaacaactccgccccattgacgcaaatgggcggtaggcgtgtacggtgggaggtctatataagcagagctcgtttagtgaaccgtcagatcgcctggatgctgatgaacttcagggtcagcttggttttggccactgactgaccaagctgactgaagttcatcaggctggctcagcactgctatgttgcctgctcttactggctggagtgaagaccagcaaaggccattcctgctgatgaacttcagggtcagcttggttttggccactgactgaccaagctgactgaagttcatcaggcctgctgagtgacagcacccctttggagccccctcccttatatctaatggaagattatgtgggcaacccggtggtagccggggtggtagagtttgacaggcaagcatgtgcgtgcagaggcgagtagtgcttgcctgtctaactcgctagtctcggcgactgtgccttctagttgccagccatctgttgtttgcccctcccccgtgccttccttgaccctggaaggtgccactcccactgtcctttcctaataaaatgaggaaattgcatcgcattgtctgagtaggtgtcattctattctggggggtggggtggggcaggacagcaagggggaggattgggaagacaatagcaggcatgctggggatgcggtgggctctatgggatacttcccgtccgccagggggacatgccggcgatgctgaaggtcgcgcgcattcccgatgaagaggccggttaccgcctgttgacctggtgggacgggcagggcgccgcccgagtcttcgcctcggcggcgggcgctctgctcatggagcgcgcgtccggggccggggaccttgcacagatagcgtggtccggccaggacgacgaggcttgcaggatcataatcagccataccacatttgtagaggttttacttgctttaaaaaacctcccacacctccccctgaacctgaaacataaaatgaatgcaattgttgttgttaacttgtttattgcagcttataatggttacaaataaagcaatagcatcacaaatttcacaaataaagcatttttttcactgcattctagttgtggtttgtccaaactcatcaatgtatcttatcaggatccccgccgccgccgccgccgccgccgccgccgccgccgccgccgccgccgccgccgccgccgccgccgccgccgccgccgccgccgccgccgccgccgccgccgccgccgccgccgccgccgccgccgccgccgccgccgccgccgccgccgccgccgccgccgccgccgccgccgccgccgccgccgccgccgccgccgccgccgccgccgccgccgccgccgccgccgccgccgccgccgccgccgccgccgccgccgccgccgccgccgccgccgccgccgccgccgccgccgccgccgtctagagtaaaggaccaagtattcagcaagttcgcttgctgaatacttggtccttgctgcctagttcaaagtcgccgtccaggcgccgcgctgttccgtttcttgctgcctcaagatcctccaggcgatctgacggttcactaaacgagctctgcttatataggcctcccaccgtacacgcctaccgcgggggtggccggggccagggcttcccacgtgcgcagcaggacgcagcgctgcctgaaactcgcgccgcgaggagagggcggggccgcggaaaggaaggggaggggctgggagggcccggagggggctgggccggggacccgggaggggtcgggacggggcggggtccgcgcggaggaggcggagctggaaggtgaaggggcaggacgggtgcccgggtccccagtccctccgccacgtggggagcgcggtcctgggcgtctgtgcccgcgaatccactgggagcccggcctggccccgacagcgcagctgctccgggcggacccgggggtctgggccgcgcttccccgcccgcgcgccgctcgcgctcccagggtgcagggacgccagcgagggccccagcggagagaggtcgaatcggcctaggctgtggggtaacccgagggaggggccataagcttatatataa

SEQ ID NO: 8 - RNA, 162 nt, Artificial sequence
  The base sequence of the adenovirus type 5 VA1 RNA
agcgggcacucuuccguggucugguggauaaauucgcaaggguaucauggcggacgaccgggguucgagccccguauccggccguccgccgugauccaugcgguuaccgcccgcgugucgaacccaggugugcgacgucagacaacgggggagugcuccuuu